European Patent Application EP 4 183 413 A1, published May 24, 2023. Title: Vaccine composition for prevention of severe acute respiratory syndrome coronavirus 2 infection. Applicant: GeneOne Life Science, Inc. The sequence listing filed with the application follows.

SEQUENCE LISTING (4 sequences)

SEQ ID NO: 1 - DNA, 3828 bp, Artificial Sequence
  pGO-1002, Spike nucleotide
atggactggacatggattctgttcctggtggcagcagcaaccagggtgcactctgtgaacctgaccacaagaacccagctgccccctgcctacaccaatagcttcacaaggggcgtgtactatccagacaaggtgtttcgcagctccgtgctgcacagcacacaggatctgtttctgcccttcttttccaacgtgacctggttccacgccatccacgtgagcggcaccaatggcacaaagaggttcgacaatcctgtgctgcccttcaacgatggcgtgtacttcgcctccaccgagaagtctaacatcatccgcggctggatctttggcaccacactggacagcaagacacagtccctgctgatcgtgaacaatgccaccaacgtggtcatcaaggtgtgcgagttccagttttgtaatgatccattcctgggcgtgtactatcacaagaacaataagtcttggatggagagcgagtttagagtgtattctagcgccaacaattgcacctttgagtacgtgtcccagcccttcctgatggacctggagggcaagcagggcaatttcaagaacctgcgggagttcgtgtttaagaatatcgatggctacttcaagatctactccaagcacacccctatcaacctggtgagagacctgccacagggcttctctgccctggagcccctggtggatctgcctatcggcatcaacatcaccaggtttcagacactgctggccctgcaccgcagctacctgacaccaggcgactcctctagcggatggaccgcaggagcagcagcctactatgtgggctatctgcagcctaggaccttcctgctgaagtacaacgagaatggcaccatcacagacgcagtggattgcgccctggaccccctgagcgagaccaagtgtacactgaagagctttaccgtggagaagggcatctatcagacaagcaatttccgggtgcagccaaccgagtccatcgtgagatttcccaatatcacaaacctgtgcccttttggcgaggtgttcaacgcaaccaggttcgccagcgtgtacgcatggaatcggaagagaatctccaactgcgtggccgactattctgtgctgtacaactctgccagcttctccacctttaagtgctatggcgtgagccccacaaagctgaatgacctgtgctttaccaacgtgtacgccgattccttcgtgatcaggggcgacgaggtgcgccagatcgcaccaggacagacaggcaagatcgccgactacaattataagctgcccgacgatttcaccggctgcgtgatcgcctggaacagcaacaatctggattccaaagtgggcggcaactacaattatctgtacaggctgtttcgcaagtccaatctgaagcctttcgagagggacatctccacagagatctaccaggccggctctaccccatgcaatggcgtggagggctttaactgttatttccccctgcagagctacggcttccagcctaccaacggcgtgggctatcagccataccgcgtggtggtgctgtcttttgagctgctgcacgcaccagcaacagtgtgcggacccaagaagagcaccaatctggtgaagaacaagtgcgtgaacttcaacttcaacggactgaccggaacaggcgtgctgaccgagtccaacaagaagttcctgccttttcagcagttcggccgggacatcgccgataccacagacgccgtgagagacccccagaccctggagatcctggacatcacaccttgctctttcggcggcgtgagcgtgatcacaccaggcaccaatacaagcaaccaggtggccgtgctgtatcaggacgtgaattgtaccgaggtgccagtggccatccacgccgatcagctgacccccacatggagggtgtacagcaccggctccaacgtgttccagacaagggcaggatgcctgatcggagcagagcacgtgaacaattcttatgagtgcgacatccccatcggcgccggcatctgtgccagctaccagacccagacaaactctcctaggagagcacggagcgtggcctctcagagcatcatcgcctataccatgtccctgggcgccgagaacagcgtggcctactctaacaatagcatcgccatccccaccaacttcacaatctccgtgaccacagagatcctgcccgtgagcatgaccaagacatctgtggactgcacaatgtatatctgtggcgattccaccgagtgctctaacctgctgctgcagtacggcagcttttgtacccagctgaatagagccctgacaggcatcgccgtggagcaggataagaacacacaggaggtgttcgcccaggtgaagcagatctacaagaccccacccatcaaggactttggcggcttcaacttcagccagatcctgcccgatccttccaagccatctaagaggagctttatcgaggacctgctgttcaacaaggtgaccctggccgatgccggcttcatcaagcagtatggcgattgcctgggcgacatcgcagcaagggacctgatctgtgcccagaagtttaatggcctgaccgtgctgcctccactgctgacagatgagatgatcgcccagtacacatctgccctgctggccggaaccatcacaagcggatggaccttcggcgcaggagccgccctgcagatcccctttgccatgcagatggcctatcggttcaacggcatcggcgtgacccagaatgtgctgtacgagaaccagaagctgatcgccaatcagtttaactccgccatcggcaagatccaggacagcctgtcctctacagcctccgccctgggcaagctgcaggatgtggtgaatcagaacgcccaggccctgaataccctggtgaagcagctgagctccaacttcggcgccatctctagcgtgctgaatgacatcctgagccggctggacaaggtggaggcagaggtgcagatcgaccggctgatcacaggcagactgcagtccctgcagacctacgtgacacagcagctgatcagggcagcagagatcagggcctctgccaatctggccgccaccaagatgagcgagtgcgtgctgggccagtccaagagagtggacttttgtggcaagggctatcacctgatgagcttcccacagtccgccccacacggagtggtgtttctgcacgtgacctacgtgcctgcccaggagaagaacttcaccacagccccagccatctgccacgatggcaaggcccactttccacgggagggcgtgttcgtgtccaacggcacccactggtttgtgacacagagaaatttctacgagccccagatcatcaccacagacaataccttcgtgagcggcaactgtgacgtggtcatcggcatcgtgaacaataccgtgtatgatcccctgcagcctgagctggactcctttaaggaggagctggataagtacttcaagaatcacacctctcctgacgtggatctgggcgacatcagcggcatcaatgcctccgtggtgaacatccagaaggagatcgacaggctgaacgaggtggccaagaatctgaacgagagcctgatcgatctgcaggagctgggcaagtatgagcagtacatcaagtggccctggtatatctggctgggcttcatcgccggcctgatcgccatcgtgatggtgaccatcatgctgtgctgtatgacatcctgctgttcttgcctgaagggctgctgtagctgtggctcctgctgtaagtttgacgaggacgattccgagcctgtgctgaagggcgtgaagctgcactacaca

SEQ ID NO: 2 - DNA, 885 bp, Artificial Sequence
  ORF3a nucleotide
atggattggacctggattctgttcctggtcgccgccgcaaccagggtgcacagcatggatctgtttatgagaatcttcacaatcggcaccgtgacactgaagcagggcgagatcaaggatgcaaccccaagcgactttgtgcgggcaaccgccacaatccctatccaggcctccctgccattcggctggctgatcgtgggagtggccctgctggccgtgtttcagtccgcctctaagatcatcacactgaagaagagatggcagctggccctgagcaagggcgtgcacttcgtgtgcaatctgctgctgctgttcgtgaccgtgtattcccacctgctgctggtggcagcaggcctggaggcacccttcctgtatctgtacgccctggtgtactttctgcagtctatcaacttcgtgcggatcatcatgagactgtggctgtgctggaagtgtcgcagcaagaatcctctgctgtatgacgccaactactttctgtgctggcacaccaactgctatgattactgtatcccttacaattccgtgacctcctctatcgtgatcacatctggcgacggcaccacatctccaatcagcgagcacgattatcagatcggcggctacaccgagaagtgggagtccggcgtgaaggactgcgtggtgctgcactcttatttcacaagcgattactatcagctgtactccacccagctgtctaccgacacaggcgtggagcacgtgacattctttatctataataagatcgtggacgagcccgaggagcacgtgcagatccacaccatcgatggcagctccggcgtggtgaaccctgtgatggagccaatctacgatgagccaaccacaaccacaagcgtgcccctgtaatga

SEQ ID NO: 3 - DNA, 3828 bp, Artificial Sequence
  pGO-1003, Spike nucleotide
atggactggacatggattctgttcctggtggcagcagcaaccagggtgcactctgtgaacctgaccacaaggacccagctgccacctgcctataccaatagcttcacaaggggcgtgtactatccagacaaggtgtttcgcagctccgtgctgcactctacacaggatctgtttctgcccttctttagcaacgtgacctggttccacgccatccacgtgagcggcaccaatggcacaaagcggttcgacaatcccgtgctgccttttaacgatggcgtgtacttcgcctctaccgagaagagcaacatcatcagaggctggatctttggcaccacactggactccaagacacagtctctgctgatcgtgaacaatgccaccaacgtggtcatcaaggtgtgcgagttccagttttgtaatgatcctttcctgggcgtgtactatcacaagaacaataagagctggatggagtccgagtttagagtgtattctagcgccaacaattgcacctttgagtacgtgtcccagccattcctgatggacctggagggcaagcagggcaatttcaagaacctgagggagttcgtgtttaagaatatcgatggctacttcaagatctactccaagcacacccctatcaacctggtgcgcgacctgccacagggcttctctgccctggagccactggtggatctgcccatcggcatcaacatcacccggtttcagacactgctggccctgcacagaagctacctgacacccggcgactcctctagcggatggaccgcaggagcagcagcctactatgtgggctatctgcagcctcggaccttcctgctgaagtacaacgagaatggcaccatcacagacgcagtggattgcgccctggaccccctgagcgagaccaagtgtacactgaagtcttttaccgtggagaagggcatctatcagacatctaatttcagggtgcagcccaccgagagcatcgtgcgctttcccaatatcacaaacctgtgcccttttggcgaggtgttcaacgccaccagattcgccagcgtgtacgcctggaatcggaagagaatctccaactgcgtggccgactattctgtgctgtacaactctgccagcttctccacctttaagtgctatggcgtgagccccacaaagctgaatgacctgtgctttaccaacgtgtacgccgattccttcgtgatcaggggcgacgaggtgagacagatcgcaccaggccagacaggcaagatcgccgactacaattataagctgcccgacgatttcaccggctgcgtgatcgcctggaactccaacaatctggattctaaagtgggcggcaactacaattatctgtaccggctgtttagaaagtccaatctgaagcctttcgagagggacatcagcacagagatctaccaggccggctccaccccatgcaatggcgtggagggctttaactgttatttccccctgcagagctacggcttccagcctaccaacggcgtgggctatcagccataccgcgtggtggtgctgtcttttgagctgctgcacgcaccagcaacagtgtgcggacctaagaagagcaccaatctggtgaagaacaagtgcgtgaacttcaacttcaacggactgaccggaacaggcgtgctgaccgagtccaacaagaagttcctgccctttcagcagttcggccgggacatcgccgataccacagacgccgtgagagaccctcagaccctggagatcctggacatcacaccatgcagcttcggcggcgtgtccgtgatcacacctggcaccaatacaagcaaccaggtggccgtgctgtatcaggacgtgaattgtaccgaggtgccagtggcaatccacgcagatcagctgacccctacatggagggtgtactccaccggctctaacgtgtttcagacaagggcaggatgcctgatcggagcagagcacgtgaacaattcctatgagtgcgacatccccatcggcgccggcatctgtgcctcttaccagacccagacaaactctcctcggagagccaggagcgtggcctctcagagcatcatcgcctataccatgtccctgggcgccgagaacagcgtggcctacagcaacaattccatcgccatccctaccaacttcacaatctccgtgaccacagagatcctgccagtgtctatgaccaagacaagcgtggactgcacaatgtatatctgtggcgattctaccgagtgcagcaacctgctgctgcagtacggcagcttttgtacccagctgaatcgcgccctgacaggaatcgcagtggagcaggataagaacacacaggaggtgttcgcccaggtgaagcagatctacaagaccccacccatcaaggactttggcggcttcaacttcagccagatcctgccagatccctctaagcccagcaagcggtcctttatcgaggacctgctgttcaacaaggtgaccctggccgatgccggcttcatcaagcagtatggcgattgcctgggcgacatcgccgccagagacctgatctgtgcccagaagtttaatggcctgaccgtgctgcctccactgctgacagatgagatgatcgcacagtacacatccgccctgctggccggcaccatcacatctggatggaccttcggcgcaggagccgccctgcagatcccctttgccatgcagatggcctataggttcaacggcatcggcgtgacccagaatgtgctgtacgagaaccagaagctgatcgccaatcagtttaactccgccatcggcaagatccaggacagcctgtcctctacagcctccgccctgggcaagctgcaggatgtggtgaatcagaacgcccaggccctgaataccctggtgaagcagctgagctccaacttcggcgccatctctagcgtgctgaatgacatcctgagccggctggacaaggtggaggcagaggtgcagatcgacaggctgatcacaggccgcctgcagtccctgcagacctacgtgacacagcagctgatccgggccgccgagatcagagcctctgccaatctggccgccaccaagatgagcgagtgcgtgctgggccagtccaagagagtggacttttgtggcaagggctatcacctgatgtccttccctcagtctgccccacacggcgtggtgtttctgcacgtgacctacgtgccagcccaggagaagaacttcaccacagcaccagccatctgccacgatggcaaggcacactttcctagggagggcgtgttcgtgtctaacggcacccactggtttgtgacacagcgcaatttctacgagccacagatcatcaccacagacaatacatttgtgagcggcaactgtgacgtggtcatcggcatcgtgaacaataccgtgtatgatccactgcagcccgagctggacagctttaaggaggagctggataagtacttcaagaatcacacctcccccgacgtggatctgggcgacatctccggcatcaatgcctctgtggtgaacatccagaaggagatcgaccgcctgaacgaggtggccaagaatctgaacgagtccctgatcgatctgcaggagctgggcaagtatgagcagtacatcaagtggccatggtatatctggctgggcttcatcgccggcctgatcgccatcgtgatggtgaccatcatgctgtgctgtatgacatcttgctgtagctgcctgaagggctgctgttcctgtggctcttgctgtaagtttgatgaggacgatagcgagcctgtgctgaagggcgtgaagctgcactacaca

SEQ ID NO: 4 - DNA, 1317 bp, Artificial Sequence
  Nucleocapsid nucleotide
atggattggacctggattctgttcctggtcgccgccgcaaccagggtgcactccatgtctgacaacggcccacagaatcagcggaacgcccccagaatcacatttggcggccctagcgattccaccggcagcaatcagaacggcgagaggagcggagcacgctccaagcagcggagaccccagggcctgcctaacaataccgcctcctggttcaccgccctgacacagcacggcaaggaggacctgaagtttccacgcggccagggcgtgcccatcaatacaaactcctctcccgacgatcagatcggctactataggagggcaaccaggagaatccggggaggcgatggcaagatgaaggacctgtcccctagatggtatttctactatctgggcacaggacctgaggcaggactgccatacggcgcaaacaaggacggaatcatctgggtggcaaccgagggcgccctgaacacaccaaaggatcacatcggcacccggaatcccgccaacaatgcagcaatcgtgctgcagctgcctcagggaaccacactgccaaagggcttctacgcagagggctctcggggaggcagccaggccagctccagatctagctccaggtctcgcaattctagcaggaacagcaccccaggctcctctaggggcacaagccctgcaaggatggcaggaaatggaggcgacgccgccctggccctgctgctgctggatcgcctgaaccagctggagagcaagatgtccggcaagggacagcagcagcagggacagaccgtgacaaagaagagcgccgcagaggcctccaagaagccaaggcagaagcgcaccgccacaaaggcctataatgtgacacaggccttcggcaggcgcggaccagagcagacccagggcaactttggcgaccaggagctgatcaggcagggaaccgattacaagcactggccacagatcgcacagttcgcaccatctgccagcgccttctttggcatgagcagaatcggcatggaggtgaccccttccggcacatggctgacctatacaggcgccatcaagctggacgataaggaccccaacttcaaggaccaggtcatcctgctgaacaagcacatcgacgcctacaagacctttccccctacagagcccaagaaggataagaagaagaaggcagacgagacacaggccctgccacagagacagaagaagcagcagaccgtgacactgctgcctgcagcagacctggacgatttctccaagcagctgcagcagtctatgagctccgccgatagcacccaggcctaatga